European Patent Application EP 4 397 687 A1, published July 10, 2024. Title: A recombinant hARSA that crosses the blood brain barrier. Applicant: Linno Pharmaceuticals lnc. The sequence listing filed with the application follows.

SEQUENCE LISTING (12 sequences)

SEQ ID NO: 1 - protein, 5 aa, synthetic construct
GNYMG

SEQ ID NO: 2 - protein, 17 aa, synthetic construct
VLYTGGGSTYYADSVKG

SEQ ID NO: 3 - protein, 19 aa, synthetic construct
ALGSARWYTSSLDARAYNI

SEQ ID NO: 4 - protein, 30 aa, synthetic construct
EVQLVESGGGLVQPGGSLRLSCAASGHAYG

SEQ ID NO: 5 - protein, 14 aa, synthetic construct
WFRQAPGKGLEGVA

SEQ ID NO: 6 - protein, 32 aa, synthetic construct
RFTISEDNSKNTVYLQMNSLRAEDTAVYYCAL

SEQ ID NO: 7 - protein, 11 aa, synthetic construct
WGQGTLVTVSS

SEQ ID NO: 8 - protein, 128 aa, synthetic construct
EVQLVESGGGLVQPGGSLRLSCAASGHAYGGNYMGWFRQAPGKGLEGVAVLYTGGGSTYYADSVKGRFTISEDNSKNTVYLQMNSLRAEDTAVYYCALALGSARWYTSSLDARAYNIWGQGTLVTVSS

SEQ ID NO: 9 - protein, 15 aa, synthetic construct
GGGGSGGGGSGGGGS

SEQ ID NO: 10 - protein, 489 aa, synthetic construct
RPPNIVLIFADDLGYGDLGCYGHPSSTTPNLDQLAAGGLRFTDFYVPVSLCTPSRAALLTGRLPVRMGMYPGVLVPSSRGGLPLEEVTVAEVLAARGYLTGMAGKWHLGVGPEGAFLPPHQGFHRFLGIPYSHDQGPCQNLTCFPPATPCDGGCDQGLVPIPLLANLSVEAQPPWLPGLEARYMAFAHDLMADAQRQDRPFFLYYASHHTHYPQFSGQSFAERSGRGPFGDSLMELDAAVGTLMTAIGDLGLLEETLVIFTADNGPETMRMSRGGCSGLLRCGKGTTYEGGVREPALAFWPGHIAPGVTHELASSLDLLPTLAALAGAPLPNVTLDGFDLSPLLLGTGKSPRQSLFFYPSYPDEVRGVFAVRTGKYKAHFFTQGSAHSDTTADPACHASSSLTAHEPPLLYDLSKDPGENYNLLGGVAGATPEVLQALKQLQLLKAQLDAAVTFGPSQVARGEDPALQICCHPGCTPRPACCHCPDPHA

SEQ ID NO: 11 - protein, 643 aa, synthetic construct
RPPNIVLIFADDLGYGDLGCYGHPSSTTPNLDQLAAGGLRFTDFYVPVSLCTPSRAALLTGRLPVRMGMYPGVLVPSSRGGLPLEEVTVAEVLAARGYLTGMAGKWHLGVGPEGAFLPPHQGFHRFLGIPYSHDQGPCQNLTCFPPATPCDGGCDQGLVPIPLLANLSVEAQPPWLPGLEARYMAFAHDLMADAQRQDRPFFLYYASHHTHYPQFSGQSFAERSGRGPFGDSLMELDAAVGTLMTAIGDLGLLEETLVIFTADNGPETMRMSRGGCSGLLRCGKGTTYEGGVREPALAFWPGHIAPGVTHELASSLDLLPTLAALAGAPLPNVTLDGFDLSPLLLGTGKSPRQSLFFYPSYPDEVRGVFAVRTGKYKAHFFTQGSAHSDTTADPACHASSSLTAHEPPLLYDLSKDPGENYNLLGGVAGATPEVLQALKQLQLLKAQLDAAVTFGPSQVARGEDPALQICCHPGCTPRPACCHCPDPHAGGGGSGGGGSGGGGSEVQLVESGGGLVQPGGSLRLSCAASGHAYGGNYMGWFRQAPGKGLEGVAVLYTGGGSTYYADSVKGRFTISEDNSKNTVYLQMNSLRAEDTAVYYCALALGSARWYTSSLDARAYNIWGQGTLVTVSSGGGGSHHHHHH

SEQ ID NO: 12 - protein, 129 aa, synthetic construct
HVQLVESGGGSVQAGGSLRLSCVASGIGHGFNNNCMGWFRQAPGKEREGVAAVYTGGGTPYYADSVKGRFTLSQDNAKNTLYLQMNGLDPEDTAMYYCVADIWRTYRCGAGDTTVFDYRGQGTLVTVSS